European Patent Specification EP 3 411 712 B1, published November 19, 2025. Title: COMPOSITIONS OF INFLUENZA HEMAGGLUTININ WITH HETEROLOGOUS EPITOPES AND/OR ALTERED MATURATION          CLEAVAGE SITES AND METHODS OF USE THEREOF. Applicant: CG Discovery, Inc. LUO, Chun. Application Not Yet Assigned. The sequence listing filed with the application follows.

SEQUENCE LISTING (62 sequences)

SEQ ID NO: 1 - protein, 566 aa, Influenza A virus
MKAILVVLLYTFATANADTLCIGYHANNSTDTVDTVLEKNVTVTHSVNLLEDKHNGKLCKLRGVAPLHLGKCNIAGWILGNPECESLSTASSWSYIVETPSSDNGTCYPGDFIDYEELREQLSSVSSFERFEIFPKTSSWPNHDSNKGVTAACPHAGAKSFYKNLIWLVKKGNSYPKLSKSYINDKGKEVLVLWGIHHPSTSADQQSLYQNADAYVFVGSSRYSKKFKPEIAIRPKVRDQEGRMNYYWTLVEPGDKITFEATGNLVVPRYAFAMERNAGSGIIISDTPVHDCNTTCQTPKGAINTSLPFQNIHPITIGKCPKYVKSTKLRLATGLRNIPSIQSRGLFGAIAGFIEGGWTGMVDGWYGYHHQNEQGSGYAADLKSTQNAIDEITNKVNSVIEKMNTQFTAVGKEFNHLEKRIENLNKKVDDGFLDIWTYNAELLVLLENERTLDYHDSNVKNLYEKVRSQLKNNAKEIGNGCFEFYHKCDNTCMESVKNGTYDYPKYSEEAKLNREEIDGVKLESTRIYQILAIYSTVASSLVLVVSLGAISFWMCSNGSLQCRICI

SEQ ID NO: 2 - protein, 20 aa, Artificial Sequence
  Synthetic
MVSAIVLYVLLAAAAHSAFA

SEQ ID NO: 3 - protein, 49 aa, Artificial Sequence
  Synthetic
GAENLYFQGGSGYIPEAPRDGQAYVRKDGEWVLLSTFLGHHHHHHHHHH

SEQ ID NO: 4 - protein, 7 aa, Artificial Sequence
  Synthetic
ENLYFQG

SEQ ID NO: 5 - protein, 29 aa, Artificial Sequence
  Synthetic
GSGYIPEAPRDGQAYVRKDGEWVLLSTFL

SEQ ID NO: 6 - protein, 10 aa, Artificial Sequence
  Synthetic
HHHHHHHHHH

SEQ ID NO: 7 - protein, 17 aa, Artificial Sequence
  Synthetic
MKAILVVLLYTFATANA

SEQ ID NO: 8 - protein, 7 aa, Artificial Sequence
  Synthetic
IPSIQSR

SEQ ID NO: 9 - protein, 581 aa, Artificial Sequence
  Synthetic
MVSAIVLYVLLAAAAHSAFADTLCIGYHANNSTDTVDTVLEKNVTVTHSVNLLEDKHNGKLCKLRGVAPLHLGKCNIAGWILGNPECESLSTASSWSYIVETPSSDNGTCYPGDFIDYEELREQLSSVSSFERFEIFPKTSSWPNHDSNKGVTAACPHAGAKSFYKNLIWLVKKGNSYPKLSKSYINDKGKEVLVLWGIHHPSTSADQQSLYQNADAYVFVGSSRYSKKFKPEIAIRPKVRDQEGRMNYYWTLVEPGDKITFEATGNLVVPRYAFAMERNAGSGIIISDTPVHDCNTTCQTPKGAINTSLPFQNIHPITIGKCPKYVKSTKLRLATGLRNIPSIQSRGLFGAIAGFIEGGWTGMVDGWYGYHHQNEQGSGYAADLKSTQNAIDEITNKVNSVIEKMNTQFTAVGKEFNHLEKRIENLNKKVDDGFLDIWTYNAELLVLLENERTLDYHDSNVKNLYEKVRSQLKNNAKEIGNGCFEFYHKCDNTCMESVKNGTYDYPKYSEEAKLNREEIDGVKLESTRIYQGAENLYFQGGSGYIPEAPRDGQAYVRKDGEWVLLSTFLGHHHHHHHHHH

SEQ ID NO: 10 - DNA, 1757 bp, Artificial Sequence
  Synthetic
ccatggtaagcgctattgttttatatgtgcttttggcggcggcggcgcattctgcctttgcggatacactgtgtattggctaccacgccaacaatagcaccgataccgtggatacagtgctggagaagaatgtgaccgtgacccactctgtgaatctgctggaggataagcacaatggcaagctgtgtaagctgagaggagttgcccctctgcacctgggcaaatgtaatattgccggctggattctgggaaatcctgaatgtgaaagcctgtctacagccagcagctggtcttatatcgtggaaacccctagcagcgacaatggcacctgttaccctggcgacttcatcgattacgaggagctgagagaacagctgtctagcgtgtccagcttcgagagattcgagatcttccctaagacaagcagctggcctaatcacgattctaataagggagtgacagccgcctgtcctcatgccggagccaagtccttttacaagaacctgatctggctggtgaagaagggcaacagctaccctaagctgtctaagagctacatcaacgacaagggcaaagaagtgctggtgctgtggggaatccaccaccctagcacaagcgccgatcagcagagcctgtaccagaatgccgatgcctatgtgtttgtgggcagcagcagatacagcaaaaagttcaagcctgaaattgccattagacccaaagtgagagatcaggaaggcagaatgaattactactggaccctggtggaacctggcgataagatcacatttgaggccaccggaaatctggtggtgcctagatatgcatttgctatggagagaaatgctggctctggcatcattatctctgatacccctgtgcacgactgtaataccacctgtcagacacctaagggcgccattaataccagcctgcccttccagaatattcaccctatcaccatcggcaagtgtcctaagtatgtgaagagcaccaagctgagactggctaccggtctgagaaatatccctagcatccagagcagaggcctgtttggagccatcgccggctttattgagggaggatggaccggaatggtggatggctggtacggctatcaccaccagaatgagcagggatccggatatgccgccgatctgaagtctacacagaacgccatcgacgagatcacaaacaaggtgaacagcgtgatcgagaagatgaacacccagtttacagctgtgggcaaggagttcaaccacctggagaagagaatcgagaacctgaacaagaaagtggacgacggcttcctggatatttggacctacaatgccgagctgctcgtgctcctggagaatgagagaaccctggactaccacgacagcaatgtgaagaacctgtacgagaaggtgagaagccagctgaagaacaatgccaaggagatcggcaacggctgctttgagttctaccacaagtgtgacaacacctgtatggagtctgtgaagaacggcacctacgactaccctaagtatagcgaggaggccaagctgaatagagaggagatcgacggcgtgaaactggaaagcacaagaatctatcagggcgctgaaaacctgtattttcagggcggttctggttacatcccggaagctccgcgtgacggtcaggcttacgttcgtaaagacggtgaatgggttctgctgtctaccttcctgggtcaccatcatcaccaccatcaccatcatcactgataaaagctt

SEQ ID NO: 11 - protein, 584 aa, Artificial Sequence
  Synthetic
MVSAIVLYVLLAAAAHSAFADTLCIGYHANNSTDTVDTVLEKNVTVTHSVNLLEDKHNGKLCKLRGVAPLHLGKCNIAGWILGNPECESLSTASSWSYIVETPSSDNGTCYPGDFIDYEELREQLSSVSSFERFEIFPKTSSWPNHDSNKGVTAACPHAGAKSFYKNLIWLVKKGNSYPKLSKSYINDKGKEVLVLWGIHHPSTSADQQSLYQNADAYVFVGSSRYSKKFKPEIAIRPKVRDQEGRMNYYWTLVEPGDKITFEATGNLVVPRYAFAMERNAGSGIIISDTPVHDCNTTCQTPKGAINTSLPFQNIHPITIGKCPKYVKSTKLRLATGLRNSPQRERRKKRGLFGAIAGFIEGGWTGMVDGWYGYHHQNEQGSGYAADLKSTQNAIDEITNKVNSVIEKMNTQFTAVGKEFNHLEKRIENLNKKVDDGFLDIWTYNAELLVLLENERTLDYHDSNVKNLYEKVRSQLKNNAKEIGNGCFEFYHKCDNTCMESVKNGTYDYPKYSEEAKLNREEIDGVKLESTRIYQGAENLYFQGGSGYIPEAPRDGQAYVRKDGEWVLLSTFLGHHHHHHHHHH

SEQ ID NO: 12 - protein, 8 aa, Artificial Sequence
  Synthetic
QRERRKKR

SEQ ID NO: 13 - DNA, 1766 bp, Artificial Sequence
  Synthetic
ccatggtaagcgctattgttttatatgtgcttttggcggcggcggcgcattctgcctttgcggatacactgtgtattggctaccacgccaacaatagcaccgataccgtggatacagtgctggagaagaatgtgaccgtgacccactctgtgaatctgctggaggataagcacaatggcaagctgtgtaagctgagaggagttgcccctctgcacctgggcaaatgtaatattgccggctggattctgggaaatcctgaatgtgaaagcctgtctacagccagcagctggtcttatatcgtggaaacccctagcagcgacaatggcacctgttaccctggcgacttcatcgattacgaggagctgagagaacagctgtctagcgtgtccagcttcgagagattcgagatcttccctaagacaagcagctggcctaatcacgattctaataagggagtgacagccgcctgtcctcatgccggagccaagtccttttacaagaacctgatctggctggtgaagaagggcaacagctaccctaagctgtctaagagctacatcaacgacaagggcaaagaagtgctggtgctgtggggaatccaccaccctagcacaagcgccgatcagcagagcctgtaccagaatgccgatgcctatgtgtttgtgggcagcagcagatacagcaaaaagttcaagcctgaaattgccattagacccaaagtgagagatcaggaaggcagaatgaattactactggaccctggtggaacctggcgataagatcacatttgaggccaccggaaatctggtggtgcctagatatgcatttgctatggagagaaatgctggctctggcatcattatctctgatacccctgtgcacgactgtaataccacctgtcagacacctaagggcgccattaataccagcctgcccttccagaatattcaccctatcaccatcggcaagtgtcctaagtatgtgaagagcaccaagctgagactggctaccggtctgagaaatagccctcagagggagagacgcaagaagagaggcctgtttggagccatcgccggctttattgagggaggatggaccggaatggtggatggctggtacggctatcaccaccagaatgagcagggatccggatatgccgccgatctgaagtctacacagaacgccatcgacgagatcacaaacaaggtgaacagcgtgatcgagaagatgaacacccagtttacagctgtgggcaaggagttcaaccacctggagaagagaatcgagaacctgaacaagaaagtggacgacggcttcctggatatttggacctacaatgccgagctgctcgtgctcctggagaatgagagaaccctggactaccacgacagcaatgtgaagaacctgtacgagaaggtgagaagccagctgaagaacaatgccaaggagatcggcaacggctgctttgagttctaccacaagtgtgacaacacctgtatggagtctgtgaagaacggcacctacgactaccctaagtatagcgaggaggccaagctgaatagagaggagatcgacggcgtgaaactggaaagcacaagaatctatcagggcgctgaaaacctgtattttcagggcggttctggttacatcccggaagctccgcgtgacggtcaggcttacgttcgtaaagacggtgaatgggttctgctgtctaccttcctgggtcaccatcatcaccaccatcaccatcatcactgataaaagctt

SEQ ID NO: 14 - protein, 581 aa, Artificial Sequence
  Synthetic
MVSAIVLYVLLAAAAHSAFADTLCIGYHANNSTDTVDTVLEKNVTVTHSVNLLEDKHNGKLCKLRGVAPLHLGKCNIAGWILGNPECESLSTASSWSYIVETPSSDNGTCYPGDFIDYEELREQLSSVSSFERFEIFPKTSSWPNHDSNKGVTAACPHAGAKSFYKNLIWLVKKGNSYPKLSKSYINDKGKEVLVLWGIHHPSTSADQQSLYQNADAYVFVGSSRYSKKFKPEIAIRPKVRDQEGRMNYYWTLVEPGDKITFEATGNLVVPRYAFAMERNAGSGIIISDTPVHDCNTTCQTPKGAINTSLPFQNIHPITIGKCPKYVKSTKLRLATGLRNIPRRRRRGLFGAIAGFIEGGWTGMVDGWYGYHHQNEQGSGYAADLKSTQNAIDEITNKVNSVIEKMNTQFTAVGKEFNHLEKRIENLNKKVDDGFLDIWTYNAELLVLLENERTLDYHDSNVKNLYEKVRSQLKNNAKEIGNGCFEFYHKCDNTCMESVKNGTYDYPKYSEEAKLNREEIDGVKLESTRIYQGAENLYFQGGSGYIPEAPRDGQAYVRKDGEWVLLSTFLGHHHHHHHHHH

SEQ ID NO: 15 - DNA, 1757 bp, Artificial Sequence
  Synthetic
ccatggtaagcgctattgttttatatgtgcttttggcggcggcggcgcattctgcctttgcggatacactgtgtattggctaccacgccaacaatagcaccgataccgtggatacagtgctggagaagaatgtgaccgtgacccactctgtgaatctgctggaggataagcacaatggcaagctgtgtaagctgagaggagttgcccctctgcacctgggcaaatgtaatattgccggctggattctgggaaatcctgaatgtgaaagcctgtctacagccagcagctggtcttatatcgtggaaacccctagcagcgacaatggcacctgttaccctggcgacttcatcgattacgaggagctgagagaacagctgtctagcgtgtccagcttcgagagattcgagatcttccctaagacaagcagctggcctaatcacgattctaataagggagtgacagccgcctgtcctcatgccggagccaagtccttttacaagaacctgatctggctggtgaagaagggcaacagctaccctaagctgtctaagagctacatcaacgacaagggcaaagaagtgctggtgctgtggggaatccaccaccctagcacaagcgccgatcagcagagcctgtaccagaatgccgatgcctatgtgtttgtgggcagcagcagatacagcaaaaagttcaagcctgaaattgccattagacccaaagtgagagatcaggaaggcagaatgaattactactggaccctggtggaacctggcgataagatcacatttgaggccaccggaaatctggtggtgcctagatatgcatttgctatggagagaaatgctggctctggcatcattatctctgatacccctgtgcacgactgtaataccacctgtcagacacctaagggcgccattaataccagcctgcccttccagaatattcaccctatcaccatcggcaagtgtcctaagtatgtgaagagcaccaagctgagactggctaccggtctgagaaatatccctaggagacgcagaagaggcctgtttggagccatcgccggctttattgagggaggatggaccggaatggtggatggctggtacggctatcaccaccagaatgagcagggatccggatatgccgccgatctgaagtctacacagaacgccatcgacgagatcacaaacaaggtgaacagcgtgatcgagaagatgaacacccagtttacagctgtgggcaaggagttcaaccacctggagaagagaatcgagaacctgaacaagaaagtggacgacggcttcctggatatttggacctacaatgccgagctgctcgtgctcctggagaatgagagaaccctggactaccacgacagcaatgtgaagaacctgtacgagaaggtgagaagccagctgaagaacaatgccaaggagatcggcaacggctgctttgagttctaccacaagtgtgacaacacctgtatggagtctgtgaagaacggcacctacgactaccctaagtatagcgaggaggccaagctgaatagagaggagatcgacggcgtgaaactggaaagcacaagaatctatcagggcgctgaaaacctgtattttcagggcggttctggttacatcccggaagctccgcgtgacggtcaggcttacgttcgtaaagacggtgaatgggttctgctgtctaccttcctgggtcaccatcatcaccaccatcaccatcatcactgataaaagctt

SEQ ID NO: 16 - protein, 585 aa, Artificial Sequence
  Synthetic
MVSAIVLYVLLAAAAHSAFADTLCIGYHANNSTDTVDTVLEKNVTVTHSVNLLEDKHNGKLCKLRGVAPLHLGKCNIAGWILGNPECESLSTASSWSYIVETPSSDNGTCYPGDFIDYEELREQLSSVSSFERFEIFPKTSSWPNHDSNKGVTAACPHAGAKSFYKNLIWLVKKGNSYPKLSKSYINDKGKEVLVLWGIHHPSTSADQQSLYQNADAYVFVGSSRYSKKFKPEIAIRPKVRDQEGRMNYYWTLVEPGDKITFEATGNLVVPRYAFAMERNAGSGIIISDTPVHDCNTTCQTPKGAINTSLPFQNIHPITIGKCPKYVKSTKLRLATGLRNIPSIQSRRRRRGLFGAIAGFIEGGWTGMVDGWYGYHHQNEQGSGYAADLKSTQNAIDEITNKVNSVIEKMNTQFTAVGKEFNHLEKRIENLNKKVDDGFLDIWTYNAELLVLLENERTLDYHDSNVKNLYEKVRSQLKNNAKEIGNGCFEFYHKCDNTCMESVKNGTYDYPKYSEEAKLNREEIDGVKLESTRIYQGAENLYFQGGSGYIPEAPRDGQAYVRKDGEWVLLSTFLGHHHHHHHHHH

SEQ ID NO: 17 - DNA, 1769 bp, Artificial Sequence
  Synthetic
ccatggtaagcgctattgttttatatgtgcttttggcggcggcggcgcattctgcctttgcggatacactgtgtattggctaccacgccaacaatagcaccgataccgtggatacagtgctggagaagaatgtgaccgtgacccactctgtgaatctgctggaggataagcacaatggcaagctgtgtaagctgagaggagttgcccctctgcacctgggcaaatgtaatattgccggctggattctgggaaatcctgaatgtgaaagcctgtctacagccagcagctggtcttatatcgtggaaacccctagcagcgacaatggcacctgttaccctggcgacttcatcgattacgaggagctgagagaacagctgtctagcgtgtccagcttcgagagattcgagatcttccctaagacaagcagctggcctaatcacgattctaataagggagtgacagccgcctgtcctcatgccggagccaagtccttttacaagaacctgatctggctggtgaagaagggcaacagctaccctaagctgtctaagagctacatcaacgacaagggcaaagaagtgctggtgctgtggggaatccaccaccctagcacaagcgccgatcagcagagcctgtaccagaatgccgatgcctatgtgtttgtgggcagcagcagatacagcaaaaagttcaagcctgaaattgccattagacccaaagtgagagatcaggaaggcagaatgaattactactggaccctggtggaacctggcgataagatcacatttgaggccaccggaaatctggtggtgcctagatatgcatttgctatggagagaaatgctggctctggcatcattatctctgatacccctgtgcacgactgtaataccacctgtcagacacctaagggcgccattaataccagcctgcccttccagaatattcaccctatcaccatcggcaagtgtcctaagtatgtgaagagcaccaagctgagactggctaccggtctgagaaatatccctagcatccagagcaggagacgcagaagaggcctgtttggagccatcgccggctttattgagggaggatggaccggaatggtggatggctggtacggctatcaccaccagaatgagcagggatccggatatgccgccgatctgaagtctacacagaacgccatcgacgagatcacaaacaaggtgaacagcgtgatcgagaagatgaacacccagtttacagctgtgggcaaggagttcaaccacctggagaagagaatcgagaacctgaacaagaaagtggacgacggcttcctggatatttggacctacaatgccgagctgctcgtgctcctggagaatgagagaaccctggactaccacgacagcaatgtgaagaacctgtacgagaaggtgagaagccagctgaagaacaatgccaaggagatcggcaacggctgctttgagttctaccacaagtgtgacaacacctgtatggagtctgtgaagaacggcacctacgactaccctaagtatagcgaggaggccaagctgaatagagaggagatcgacggcgtgaaactggaaagcacaagaatctatcagggcgctgaaaacctgtattttcagggcggttctggttacatcccggaagctccgcgtgacggtcaggcttacgttcgtaaagacggtgaatgggttctgctgtctaccttcctgggtcaccatcatcaccaccatcaccatcatcactgataaaagctt

SEQ ID NO: 18 - protein, 581 aa, Artificial Sequence
  Synthetic
MVSAIVLYVLLAAAAHSAFADTLCIGYHANNSTDTVDTVLEKNVTVTHSVNLLEDKHNGKLCKLRGVAPLHLGKCNIAGWILGNPECESLSTASSWSYIVETPSSDNGTCYPGDFIDYEELREQLSSVSSFERFEIFPKTSSWPNHDSNKGVTAACPHAGAKSFYKNLIWLVKKGNSYPKLSKSYINDKGKEVLVLWGIHHPSTSADQQSLYQNADAYVFVGSSRYSKKFKPEIAIRPKVRDQEGRMNYYWTLVEPGDKITFEATGNLVVPRYAFAMERNAGSGIIISDTPVHDCNTTCQTPKGAINTSLPFQNIHPITIGKCPKYVKSTKLRLATGLRNIENLYFQGLFGAIAGFIEGGWTGMVDGWYGYHHQNEQGSGYAADLKSTQNAIDEITNKVNSVIEKMNTQFTAVGKEFNHLEKRIENLNKKVDDGFLDIWTYNAELLVLLENERTLDYHDSNVKNLYEKVRSQLKNNAKEIGNGCFEFYHKCDNTCMESVKNGTYDYPKYSEEAKLNREEIDGVKLESTRIYQGAENLYFQGGSGYIPEAPRDGQAYVRKDGEWVLLSTFLGHHHHHHHHHH

SEQ ID NO: 19 - DNA, 1757 bp, Artificial Sequence
  Synthetic
ccatggtaagcgctattgttttatatgtgcttttggcggcggcggcgcattctgcctttgcggatacactgtgtattggctaccacgccaacaatagcaccgataccgtggatacagtgctggagaagaatgtgaccgtgacccactctgtgaatctgctggaggataagcacaatggcaagctgtgtaagctgagaggagttgcccctctgcacctgggcaaatgtaatattgccggctggattctgggaaatcctgaatgtgaaagcctgtctacagccagcagctggtcttatatcgtggaaacccctagcagcgacaatggcacctgttaccctggcgacttcatcgattacgaggagctgagagaacagctgtctagcgtgtccagcttcgagagattcgagatcttccctaagacaagcagctggcctaatcacgattctaataagggagtgacagccgcctgtcctcatgccggagccaagtccttttacaagaacctgatctggctggtgaagaagggcaacagctaccctaagctgtctaagagctacatcaacgacaagggcaaagaagtgctggtgctgtggggaatccaccaccctagcacaagcgccgatcagcagagcctgtaccagaatgccgatgcctatgtgtttgtgggcagcagcagatacagcaaaaagttcaagcctgaaattgccattagacccaaagtgagagatcaggaaggcagaatgaattactactggaccctggtggaacctggcgataagatcacatttgaggccaccggaaatctggtggtgcctagatatgcatttgctatggagagaaatgctggctctggcatcattatctctgatacccctgtgcacgactgtaataccacctgtcagacacctaagggcgccattaataccagcctgcccttccagaatattcaccctatcaccatcggcaagtgtcctaagtatgtgaagagcaccaagctgagactggctaccggtctgagaaatatcgaaaacctgtattttcaaggcctgtttggagccatcgccggctttattgagggaggatggaccggaatggtggatggctggtacggctatcaccaccagaatgagcagggatccggatatgccgccgatctgaagtctacacagaacgccatcgacgagatcacaaacaaggtgaacagcgtgatcgagaagatgaacacccagtttacagctgtgggcaaggagttcaaccacctggagaagagaatcgagaacctgaacaagaaagtggacgacggcttcctggatatttggacctacaatgccgagctgctcgtgctcctggagaatgagagaaccctggactaccacgacagcaatgtgaagaacctgtacgagaaggtgagaagccagctgaagaacaatgccaaggagatcggcaacggctgctttgagttctaccacaagtgtgacaacacctgtatggagtctgtgaagaacggcacctacgactaccctaagtatagcgaggaggccaagctgaatagagaggagatcgacggcgtgaaactggaaagcacaagaatctatcagggcgctgaaaacctgtattttcagggcggttctggttacatcccggaagctccgcgtgacggtcaggcttacgttcgtaaagacggtgaatgggttctgctgtctaccttcctgggtcaccatcatcaccaccatcaccatcatcactgataaaagctt

SEQ ID NO: 20 - protein, 582 aa, Artificial Sequence
  Synthetic
MVSAIVLYVLLAAAAHSAFADTLCIGYHANNSTDTVDTVLEKNVTVTHSVNLLEDKHNGKLCKLRGVAPLHLGKCNIAGWILGNPECESLSTASSWSYIVETPSSDNGTCYPGDFIDYEELREQLSSVSSFERFEIFPKTSSWPNHDSNKGVTAACPHAGAKSFYKNLIWLVKKGNSYPKLSKSYINDKGKEVLVLWGIHHPSTSADQQSLYQNADAYVFVGSSRYSKKFKPEIAIRPKVRDQEGRMNYYWTLVEPGDKITFEATGNLVVPRYAFAMERNAGSGIIISDTPVHDCNTTCQTPKGAINTSLPFQNIHPITIGKCPKYVKSTKLRLATGLRNSPENLYFQGLFGAIAGFIEGGWTGMVDGWYGYHHQNEQGSGYAADLKSTQNAIDEITNKVNSVIEKMNTQFTAVGKEFNHLEKRIENLNKKVDDGFLDIWTYNAELLVLLENERTLDYHDSNVKNLYEKVRSQLKNNAKEIGNGCFEFYHKCDNTCMESVKNGTYDYPKYSEEAKLNREEIDGVKLESTRIYQGAENLYFQGGSGYIPEAPRDGQAYVRKDGEWVLLSTFLGHHHHHHHHHH

SEQ ID NO: 21 - DNA, 1760 bp, Artificial Sequence
  Synthetic
ccatggtaagcgctattgttttatatgtgcttttggcggcggcggcgcattctgcctttgcggatacactgtgtattggctaccacgccaacaatagcaccgataccgtggatacagtgctggagaagaatgtgaccgtgacccactctgtgaatctgctggaggataagcacaatggcaagctgtgtaagctgagaggagttgcccctctgcacctgggcaaatgtaatattgccggctggattctgggaaatcctgaatgtgaaagcctgtctacagccagcagctggtcttatatcgtggaaacccctagcagcgacaatggcacctgttaccctggcgacttcatcgattacgaggagctgagagaacagctgtctagcgtgtccagcttcgagagattcgagatcttccctaagacaagcagctggcctaatcacgattctaataagggagtgacagccgcctgtcctcatgccggagccaagtccttttacaagaacctgatctggctggtgaagaagggcaacagctaccctaagctgtctaagagctacatcaacgacaagggcaaagaagtgctggtgctgtggggaatccaccaccctagcacaagcgccgatcagcagagcctgtaccagaatgccgatgcctatgtgtttgtgggcagcagcagatacagcaaaaagttcaagcctgaaattgccattagacccaaagtgagagatcaggaaggcagaatgaattactactggaccctggtggaacctggcgataagatcacatttgaggccaccggaaatctggtggtgcctagatatgcatttgctatggagagaaatgctggctctggcatcattatctctgatacccctgtgcacgactgtaataccacctgtcagacacctaagggcgccattaataccagcctgcccttccagaatattcaccctatcaccatcggcaagtgtcctaagtatgtgaagagcaccaagctgagactggctaccggtctgagaaatagccctgaaaacctgtattttcaaggcctgtttggagccatcgccggctttattgagggaggatggaccggaatggtggatggctggtacggctatcaccaccagaatgagcagggatccggatatgccgccgatctgaagtctacacagaacgccatcgacgagatcacaaacaaggtgaacagcgtgatcgagaagatgaacacccagtttacagctgtgggcaaggagttcaaccacctggagaagagaatcgagaacctgaacaagaaagtggacgacggcttcctggatatttggacctacaatgccgagctgctcgtgctcctggagaatgagagaaccctggactaccacgacagcaatgtgaagaacctgtacgagaaggtgagaagccagctgaagaacaatgccaaggagatcggcaacggctgctttgagttctaccacaagtgtgacaacacctgtatggagtctgtgaagaacggcacctacgactaccctaagtatagcgaggaggccaagctgaatagagaggagatcgacggcgtgaaactggaaagcacaagaatctatcagggcgctgaaaacctgtattttcagggcggttctggttacatcccggaagctccgcgtgacggtcaggcttacgttcgtaaagacggtgaatgggttctgctgtctaccttcctgggtcaccatcatcaccaccatcaccatcatcactgataaaagctt

SEQ ID NO: 22 - protein, 584 aa, Artificial Sequence
  Synthetic
MVSAIVLYVLLAAAAHSAFADTLCIGYHANNSTDTVDTVLEKNVTVTHSVNLLEDKHNGKLCKLRGVAPLHLGKCNIAGWILGNPECESLSTASSWSYIVETPSSDNGTCYPGDFIDYEELREQLSSVSSFERFEIFPKTSSWPNHDSNKGVTAACPHAGAKSFYKNLIWLVKKGNSYPKLSKSYINDKGKEVLVLWGIHHPSTSADQQSLYQNADAYVFVGSSRYSKKFKPEIAIRPKVRDQEGRMNYYWTLVEPGDKITFEATGNLVVPRYAFAMERNAGSGIIISDTPVHDCNTTCQTPKGAINTSLPFQNIHPITIGKCPKYVKSTKLRLATGLRNIPSIENLYFQGLFGAIAGFIEGGWTGMVDGWYGYHHQNEQGSGYAADLKSTQNAIDEITNKVNSVIEKMNTQFTAVGKEFNHLEKRIENLNKKVDDGFLDIWTYNAELLVLLENERTLDYHDSNVKNLYEKVRSQLKNNAKEIGNGCFEFYHKCDNTCMESVKNGTYDYPKYSEEAKLNREEIDGVKLESTRIYQGAENLYFQGGSGYIPEAPRDGQAYVRKDGEWVLLSTFLGHHHHHHHHHH

SEQ ID NO: 23 - DNA, 1766 bp, Artificial Sequence
  Synthetic
ccatggtaagcgctattgttttatatgtgcttttggcggcggcggcgcattctgcctttgcggatacactgtgtattggctaccacgccaacaatagcaccgataccgtggatacagtgctggagaagaatgtgaccgtgacccactctgtgaatctgctggaggataagcacaatggcaagctgtgtaagctgagaggagttgcccctctgcacctgggcaaatgtaatattgccggctggattctgggaaatcctgaatgtgaaagcctgtctacagccagcagctggtcttatatcgtggaaacccctagcagcgacaatggcacctgttaccctggcgacttcatcgattacgaggagctgagagaacagctgtctagcgtgtccagcttcgagagattcgagatcttccctaagacaagcagctggcctaatcacgattctaataagggagtgacagccgcctgtcctcatgccggagccaagtccttttacaagaacctgatctggctggtgaagaagggcaacagctaccctaagctgtctaagagctacatcaacgacaagggcaaagaagtgctggtgctgtggggaatccaccaccctagcacaagcgccgatcagcagagcctgtaccagaatgccgatgcctatgtgtttgtgggcagcagcagatacagcaaaaagttcaagcctgaaattgccattagacccaaagtgagagatcaggaaggcagaatgaattactactggaccctggtggaacctggcgataagatcacatttgaggccaccggaaatctggtggtgcctagatatgcatttgctatggagagaaatgctggctctggcatcattatctctgatacccctgtgcacgactgtaataccacctgtcagacacctaagggcgccattaataccagcctgcccttccagaatattcaccctatcaccatcggcaagtgtcctaagtatgtgaagagcaccaagctgagactggctaccggtctgagaaatatccctagcatcgaaaacctgtattttcaaggcctgtttggagccatcgccggctttattgagggaggatggaccggaatggtggatggctggtacggctatcaccaccagaatgagcagggatccggatatgccgccgatctgaagtctacacagaacgccatcgacgagatcacaaacaaggtgaacagcgtgatcgagaagatgaacacccagtttacagctgtgggcaaggagttcaaccacctggagaagagaatcgagaacctgaacaagaaagtggacgacggcttcctggatatttggacctacaatgccgagctgctcgtgctcctggagaatgagagaaccctggactaccacgacagcaatgtgaagaacctgtacgagaaggtgagaagccagctgaagaacaatgccaaggagatcggcaacggctgctttgagttctaccacaagtgtgacaacacctgtatggagtctgtgaagaacggcacctacgactaccctaagtatagcgaggaggccaagctgaatagagaggagatcgacggcgtgaaactggaaagcacaagaatctatcagggcgctgaaaacctgtattttcagggcggttctggttacatcccggaagctccgcgtgacggtcaggcttacgttcgtaaagacggtgaatgggttctgctgtctaccttcctgggtcaccatcatcaccaccatcaccatcatcactgataaaagctt

SEQ ID NO: 24 - protein, 585 aa, Artificial Sequence
  Synthetic
MVSAIVLYVLLAAAAHSAFADTLCIGYHANNSTDTVDTVLEKNVTVTHSVNLLEDKHNGKLCKLRGVAPLHLGKCNIAGWILGNPECESLSTASSWSYIVETPSSDNGTCYPGDFIDYEELREQLSSVSSFERFEIFPKTSSWPNHDSNKGVTAACPHAGAKSFYKNLIWLVKKGNSYPKLSKSYINDKGKEVLVLWGIHHPSTSADQQSLYQNADAYVFVGSSRYSKKFKPEGMIDYEGTGQAAGRMNYYWTLVEPGDKITFEATGNLVVPRYAFAMERNAGSGIIISDTPVHDCNTTCQTPKGAINTSLPFQNIHPITIGKCPKYVKSTKLRLATGLRNSPQRERRKKRGLFGAIAGFIEGGWTGMVDGWYGYHHQNEQGSGYAADLKSTQNAIDEITNKVNSVIEKMNTQFTAVGKEFNHLEKRIENLNKKVDDGFLDIWTYNAELLVLLENERTLDYHDSNVKNLYEKVRSQLKNNAKEIGNGCFEFYHKCDNTCMESVKNGTYDYPKYSEEAKLNREEIDGVKLESTRIYQGAENLYFQGGSGYIPEAPRDGQAYVRKDGEWVLLSTFLGHHHHHHHHHH

SEQ ID NO: 25 - protein, 5 aa, Artificial Sequence
  Synthetic
EGMID

SEQ ID NO: 26 - protein, 7 aa, Artificial Sequence
  Synthetic
EGTGQAA

SEQ ID NO: 27 - protein, 13 aa, Artificial Sequence
  Synthetic
EGMIDYEGTGQAA

SEQ ID NO: 28 - DNA, 1770 bp, Artificial Sequence
  Synthetic
ccatggtaagcgctattgttttatatgtgcttttggcggcggcggcgcattctgcctttgcggatacactgtgtattggctaccacgccaacaatagcaccgataccgtggatacagtgctggagaagaatgtgaccgtgacccactctgtgaatctgctggaggataagcacaatggcaagctgtgtaagctgagaggagttgcccctctgcacctgggcaaatgtaatattgccggctggattctgggaaatcctgaatgtgaaagcctgtctacagccagcagctggtcttatatcgtggaaacccctagcagcgacaatggcacctgttaccctggcgacttcatcgattacgaggagctgagagaacagctgtctagcgtgtccagcttcgagagattcgagatcttccctaagacaagcagctggcctaatcacgattctaataagggagtgacagccgcctgtcctcatgccggagccaagtccttttacaagaacctgatctggctggtgaagaagggcaacagctaccctaagctgtctaagagctacatcaacgacaagggcaaagaagtgctggtgctgtggggaatccaccaccctagcacaagcgccgatcagcagagcctgtaccagaatgccgatgcctatgtgtttgtgggcagcagcagatacagcaaaaagttcaagcctgaaggcatgattgattacgaaggcacaggccaggcagccggcagaatgaattactactggaccctggtggaacctggcgataagatcacatttgaggccaccggaaatctggtggtgcctagatatgcatttgctatggagagaaatgctggctctggcatcattatctctgatacccctgtgcacgactgtaataccacctgtcagacacctaagggcgccattaataccagcctgcccttccagaatattcaccctatcaccatcggcaagtgtcctaagtatgtgaagagcaccaagctgagactggctaccggtctgagaaatagccctcagagggagagacgcaagaagagaggcctgtttggagccatcgccggctttattgagggaggatggaccggaatggtggatggctggtacggctatcaccaccagaatgagcagggatccggatatgccgccgatctgaagtctacacagaacgccatcgacgagatcacaaacaaggtgaacagcgtgatcgagaagatgaacacccagtttacagctgtgggcaaggagttcaaccacctggagaagagaatcgagaacctgaacaagaaagtggacgacggcttcctggatatttggacctacaatgccgagctgctcgtgctcctggagaatgagagaaccctggactaccacgacagcaatgtgaagaacctgtacgagaaggtgagaagccagctgaagaacaatgccaaggagatcggcaacggctgctttgagttctaccacaagtgtgacaacacctgtatggagtctgtgaagaacggcacctacgactaccctaagtatagcgaggaggccaagctgaatagagaggagatcgacggcgtgaaactggaaagcacaagaatctatcagggcgctgaaaacctgtattttcagggcggttctggttacatcccggaagctccgcgtgacggtcaggcttacgttcgtaaagacggtgaatgggttctgctgtctaccttcctgggtcaccatcatcaccaccatcaccatcatcactgataaaaagctt

SEQ ID NO: 29 - protein, 583 aa, Artificial Sequence
  Synthetic
MVSAIVLYVLLAAAAHSAFADTLCIGYHANNSTDTVDTVLEKNVTVTHSVNLLEDKHNGKLCKLRGVAPLHLGKCNIAGWILGNPECESLSTASSWSYIVETPSSDNGTCYPGDFIDYEELREQLSSVSSFERFEIFPKTSSWPNHDSNKGVTAACPHAGAKSFYKNLIWLVKKGNSYPKLSKSYINDKGKEVLVLWGIHHPSTSADQQSLYQNADAYVFVGSSRYSKKFKPEGMIDYEGTGQAAGRMNYYWTLVEPGDKITFEATGNLVVPRYAFAMERNAGSGIIISDTPVHDCNTTCQTPKGAINTSLPFQNIHPITIGKCPKYVKSTKLRLATGLRNSPENLYFQGLFGAIAGFIEGGWTGMVDGWYGYHHQNEQGSGYAADLKSTQNAIDEITNKVNSVIEKMNTQFTAVGKEFNHLEKRIENLNKKVDDGFLDIWTYNAELLVLLENERTLDYHDSNVKNLYEKVRSQLKNNAKEIGNGCFEFYHKCDNTCMESVKNGTYDYPKYSEEAKLNREEIDGVKLESTRIYQGAENLYFQGGSGYIPEAPRDGQAYVRKDGEWVLLSTFLGHHHHHHHHHH

SEQ ID NO: 30 - DNA, 1763 bp, Artificial Sequence
  Synthetic
ccatggtaagcgctattgttttatatgtgcttttggcggcggcggcgcattctgcctttgcggatacactgtgtattggctaccacgccaacaatagcaccgataccgtggatacagtgctggagaagaatgtgaccgtgacccactctgtgaatctgctggaggataagcacaatggcaagctgtgtaagctgagaggagttgcccctctgcacctgggcaaatgtaatattgccggctggattctgggaaatcctgaatgtgaaagcctgtctacagccagcagctggtcttatatcgtggaaacccctagcagcgacaatggcacctgttaccctggcgacttcatcgattacgaggagctgagagaacagctgtctagcgtgtccagcttcgagagattcgagatcttccctaagacaagcagctggcctaatcacgattctaataagggagtgacagccgcctgtcctcatgccggagccaagtccttttacaagaacctgatctggctggtgaagaagggcaacagctaccctaagctgtctaagagctacatcaacgacaagggcaaagaagtgctggtgctgtggggaatccaccaccctagcacaagcgccgatcagcagagcctgtaccagaatgccgatgcctatgtgtttgtgggcagcagcagatacagcaaaaagttcaagcctgaaggcatgattgattacgaaggcacaggccaggcagccggcagaatgaattactactggaccctggtggaacctggcgataagatcacatttgaggccaccggaaatctggtggtgcctagatatgcatttgctatggagagaaatgctggctctggcatcattatctctgatacccctgtgcacgactgtaataccacctgtcagacacctaagggcgccattaataccagcctgcccttccagaatattcaccctatcaccatcggcaagtgtcctaagtatgtgaagagcaccaagctgagactggctaccggtctgagaaatagccctgaaaacctgtattttcaaggcctgtttggagccatcgccggctttattgagggaggatggaccggaatggtggatggctggtacggctatcaccaccagaatgagcagggatccggatatgccgccgatctgaagtctacacagaacgccatcgacgagatcacaaacaaggtgaacagcgtgatcgagaagatgaacacccagtttacagctgtgggcaaggagttcaaccacctggagaagagaatcgagaacctgaacaagaaagtggacgacggcttcctggatatttggacctacaatgccgagctgctcgtgctcctggagaatgagagaaccctggactaccacgacagcaatgtgaagaacctgtacgagaaggtgagaagccagctgaagaacaatgccaaggagatcggcaacggctgctttgagttctaccacaagtgtgacaacacctgtatggagtctgtgaagaacggcacctacgactaccctaagtatagcgaggaggccaagctgaatagagaggagatcgacggcgtgaaactggaaagcacaagaatctatcagggcgctgaaaacctgtattttcagggcggttctggttacatcccggaagctccgcgtgacggtcaggcttacgttcgtaaagacggtgaatgggttctgctgtctaccttcctgggtcaccatcatcaccaccatcaccatcatcactgataaaagctt

SEQ ID NO: 31 - protein, 590 aa, Artificial Sequence
  Synthetic
MVSAIVLYVLLAAAAHSAFADTLCIGYHANNSTDTVDTVLEKNVTVTHSVNLLEDKHNGKLCKLRGVAPLHLGKCNIAGWILGNPECESLSTASSWSYIVETPSSDNGTCYPGDFIDYEELREQLSSVSSFERFEIFPKTSSWPNHDSNKGVTAACPHAGAKSFYKNLIWLVEGMIDYEGTGQAAYPKLSKSYINDKGKEVLVLWGIHHPSTSADQQSLYQNADAYVFVGSSRYSKKFKPEIAIRPKVRDQEGRMNYYWTLVEPGDKITFEATGNLVVPRYAFAMERNAGSGIIISDTPVHDCNTTCQTPKGAINTSLPFQNIHPITIGKCPKYVKSTKLRLATGLRNSPENLYFQGLFGAIAGFIEGGWTGMVDGWYGYHHQNEQGSGYAADLKSTQNAIDEITNKVNSVIEKMNTQFTAVGKEFNHLEKRIENLNKKVDDGFLDIWTYNAELLVLLENERTLDYHDSNVKNLYEKVRSQLKNNAKEIGNGCFEFYHKCDNTCMESVKNGTYDYPKYSEEAKLNREEIDGVKLESTRIYQGAENLYFQGGSGYIPEAPRDGQAYVRKDGEWVLLSTFLGHHHHHHHHHH

SEQ ID NO: 32 - DNA, 1785 bp, Artificial Sequence
  Synthetic
ccatggtaagcgctattgttttatatgtgcttttggcggcggcggcgcattctgcctttgcggatacactgtgtattggctaccacgccaacaatagcaccgataccgtggatacagtgctggagaagaatgtgaccgtgacccactctgtgaatctgctggaggataagcacaatggcaagctgtgtaagctgagaggagttgcccctctgcacctgggcaaatgtaatattgccggctggattctgggaaatcctgaatgtgaaagcctgtctacagccagcagctggtcttatatcgtggaaacccctagcagcgacaatggcacctgttaccctggcgacttcatcgattacgaggagctgagagaacagctgtctagcgtgtccagcttcgagagattcgagatcttccctaagacaagcagctggcctaatcacgattctaataagggagtgacagccgcctgtcctcatgccggagccaagtccttttacaagaacctgatctggctggtggaaggcatgattgattacgaaggcacaggccaggcagcctaccctaagctgtctaagagctacatcaacgacaagggcaaagaagtgctggtgctgtggggaatccaccaccctagcacaagcgccgatcagcagagcctgtaccagaatgccgatgcctatgtgtttgtgggcagcagcagatacagcaaaaagttcaagcctgaaattgccattagacccaaagtgagagatcaggaaggcagaatgaattactactggaccctggtggaacctggcgataagatcacatttgaggccaccggaaatctggtggtgcctagatatgcatttgctatggagagaaatgctggctctggcatcattatctctgatacccctgtgcacgactgtaataccacctgtcagacacctaagggcgccattaataccagcctgcccttccagaatattcaccctatcaccatcggcaagtgtcctaagtatgtgaagagcaccaagctgagactggctaccggtctgagaaatagccctgaaaacctgtattttcaaggcctgtttggagccatcgccggctttattgagggaggatggaccggaatggtggatggctggtacggctatcaccaccagaatgagcagggatccggatatgccgccgatctgaagtctacacagaacgccatcgacgagatcacaaacaaggtgaacagcgtgatcgagaagatgaacacccagtttacagctgtgggcaaggagttcaaccacctggagaagagaatcgagaacctgaacaagaaagtggacgacggcttcctggatatttggacctacaatgccgagctgctcgtgctcctggagaatgagagaaccctggactaccacgacagcaatgtgaagaacctgtacgagaaggtgagaagccagctgaagaacaatgccaaggagatcggcaacggctgctttgagttctaccacaagtgtgacaacacctgtatggagtctgtgaagaacggcacctacgactaccctaagtatagcgaggaggccaagctgaatagagaggagatcgacggcgtgaaactggaaagcacaagaatctatcagggcgctgaaaacctgtattttcagggcggttctggttacatcccggaagctccgcgtgacggtcaggcttacgttcgtaaagacggtgaatgggttctgctgtctaccttcctgggtcaccatcatcaccaccatcaccatcatcactgataaaaagctt

SEQ ID NO: 33 - protein, 591 aa, Artificial Sequence
  Synthetic
MVSAIVLYVLLAAAAHSAFADTLCIGYHANNSTDTVDTVLEKNVTVTHSVNLLEDKHNGKLCKLRGVAPLHLGKCNIAGWILGNPECESLSTASSWSYIVETPSSDNGTCYPGDFIDYEELREQLSSVSSFERFEIFPEGMIDYEGTGQAAWPNHDSNKGVTAACPHAGAKSFYKNLIWLVKKGNSYPKLSKSYINDKGKEVLVLWGIHHPSTSADQQSLYQNADAYVFVGSSRYSKKFKPEIAIRPKVRDQEGRMNYYWTLVEPGDKITFEATGNLVVPRYAFAMERNAGSGIIISDTPVHDCNTTCQTPKGAINTSLPFQNIHPITIGKCPKYVKSTKLRLATGLRNSPENLYFQGLFGAIAGFIEGGWTGMVDGWYGYHHQNEQGSGYAADLKSTQNAIDEITNKVNSVIEKMNTQFTAVGKEFNHLEKRIENLNKKVDDGFLDIWTYNAELLVLLENERTLDYHDSNVKNLYEKVRSQLKNNAKEIGNGCFEFYHKCDNTCMESVKNGTYDYPKYSEEAKLNREEIDGVKLESTRIYQGAENLYFQGGSGYIPEAPRDGQAYVRKDGEWVLLSTFLGHHHHHHHHHH

SEQ ID NO: 34 - DNA, 1787 bp, Artificial Sequence
  Synthetic
ccatggtaagcgctattgttttatatgtgcttttggcggcggcggcgcattctgcctttgcggatacactgtgtattggctaccacgccaacaatagcaccgataccgtggatacagtgctggagaagaatgtgaccgtgacccactctgtgaatctgctggaggataagcacaatggcaagctgtgtaagctgagaggagttgcccctctgcacctgggcaaatgtaatattgccggctggattctgggaaatcctgaatgtgaaagcctgtctacagccagcagctggtcttatatcgtggaaacccctagcagcgacaatggcacctgttaccctggcgacttcatcgattacgaggagctgagagaacagctgtctagcgtgtccagcttcgagagattcgagatcttccctgaaggcatgattgattacgaaggcacaggccaggcagcctggcctaatcacgattctaataagggagtgacagccgcctgtcctcatgccggagccaagtccttttacaagaacctgatctggctggtgaagaagggcaacagctaccctaagctgtctaagagctacatcaacgacaagggcaaagaagtgctggtgctgtggggaatccaccaccctagcacaagcgccgatcagcagagcctgtaccagaatgccgatgcctatgtgtttgtgggcagcagcagatacagcaaaaagttcaagcctgaaattgccattagacccaaagtgagagatcaggaaggcagaatgaattactactggaccctggtggaacctggcgataagatcacatttgaggccaccggaaatctggtggtgcctagatatgcatttgctatggagagaaatgctggctctggcatcattatctctgatacccctgtgcacgactgtaataccacctgtcagacacctaagggcgccattaataccagcctgcccttccagaatattcaccctatcaccatcggcaagtgtcctaagtatgtgaagagcaccaagctgagactggctaccggtctgagaaatagccctgaaaacctgtattttcaaggcctgtttggagccatcgccggctttattgagggaggatggaccggaatggtggatggctggtacggctatcaccaccagaatgagcagggatccggatatgccgccgatctgaagtctacacagaacgccatcgacgagatcacaaacaaggtgaacagcgtgatcgagaagatgaacacccagtttacagctgtgggcaaggagttcaaccacctggagaagagaatcgagaacctgaacaagaaagtggacgacggcttcctggatatttggacctacaatgccgagctgctcgtgctcctggagaatgagagaaccctggactaccacgacagcaatgtgaagaacctgtacgagaaggtgagaagccagctgaagaacaatgccaaggagatcggcaacggctgctttgagttctaccacaagtgtgacaacacctgtatggagtctgtgaagaacggcacctacgactaccctaagtatagcgaggaggccaagctgaatagagaggagatcgacggcgtgaaactggaaagcacaagaatctatcagggcgctgaaaacctgtattttcagggcggttctggttacatcccggaagctccgcgtgacggtcaggcttacgttcgtaaagacggtgaatgggttctgctgtctaccttcctgggtcaccatcatcaccaccatcaccatcatcactgataaaagctt

SEQ ID NO: 35 - protein, 586 aa, Artificial Sequence
  Synthetic
MVSAIVLYVLLAAAAHSAFADTLCIGYHANNSTDTVDTVLEKNVTVTHSVNLLEDKHNGKLCKLRGVAPLHLGKCNIAGWILGNPECESLSTASSWSYIVETPSSDNGTCYPGDFIDYEELREQLSSVSSFERFEIFPKTSSWPNHDSNKGVTAACPHAGAKSFYKNLIWLVKKGNSYPKLSKSYINDKGKEVLVLWGIHHPSTSADQQSLYQNADAYVFVGSSRYSKKFKPEIAIGIFGAIAGFIEGGRMNYYWTLVEPGDKITFEATGNLVVPRYAFAMERNAGSGIIISDTPVHDCNTTCQTPKGAINTSLPFQNIHPITIGKCPKYVKSTKLRLATGLRNSPENLYFQGLFGAIAGFIEGGWTGMVDGWYGYHHQNEQGSGYAADLKSTQNAIDEITNKVNSVIEKMNTQFTAVGKEFNHLEKRIENLNKKVDDGFLDIWTYNAELLVLLENERTLDYHDSNVKNLYEKVRSQLKNNAKEIGNGCFEFYHKCDNTCMESVKNGTYDYPKYSEEAKLNREEIDGVKLESTRIYQGAENLYFQGGSGYIPEAPRDGQAYVRKDGEWVLLSTFLGHHHHHHHHHH

SEQ ID NO: 36 - protein, 12 aa, Artificial Sequence
  Synthetic
GIFGAIAGFIEG

SEQ ID NO: 37 - DNA, 1772 bp, Artificial Sequence
  Synthetic
ccatggtaagcgctattgttttatatgtgcttttggcggcggcggcgcattctgcctttgcggatacactgtgtattggctaccacgccaacaatagcaccgataccgtggatacagtgctggagaagaatgtgaccgtgacccactctgtgaatctgctggaggataagcacaatggcaagctgtgtaagctgagaggagttgcccctctgcacctgggcaaatgtaatattgccggctggattctgggaaatcctgaatgtgaaagcctgtctacagccagcagctggtcttatatcgtggaaacccctagcagcgacaatggcacctgttaccctggcgacttcatcgattacgaggagctgagagaacagctgtctagcgtgtccagcttcgagagattcgagatcttccctaagacaagcagctggcctaatcacgattctaataagggagtgacagccgcctgtcctcatgccggagccaagtccttttacaagaacctgatctggctggtgaagaagggcaacagctaccctaagctgtctaagagctacatcaacgacaagggcaaagaagtgctggtgctgtggggaatccaccaccctagcacaagcgccgatcagcagagcctgtaccagaatgccgatgcctatgtgtttgtgggcagcagcagatacagcaaaaagttcaagcctgaaattgccattggcattttcggcgctatcgccggcttcattgagggaggcagaatgaattactactggaccctggtggaacctggcgataagatcacatttgaggccaccggaaatctggtggtgcctagatatgcatttgctatggagagaaatgctggctctggcatcattatctctgatacccctgtgcacgactgtaataccacctgtcagacacctaagggcgccattaataccagcctgcccttccagaatattcaccctatcaccatcggcaagtgtcctaagtatgtgaagagcaccaagctgagactggctaccggtctgagaaatagccctgaaaacctgtattttcaaggcctgtttggagccatcgccggctttattgagggaggatggaccggaatggtggatggctggtacggctatcaccaccagaatgagcagggatccggatatgccgccgatctgaagtctacacagaacgccatcgacgagatcacaaacaaggtgaacagcgtgatcgagaagatgaacacccagtttacagctgtgggcaaggagttcaaccacctggagaagagaatcgagaacctgaacaagaaagtggacgacggcttcctggatatttggacctacaatgccgagctgctcgtgctcctggagaatgagagaaccctggactaccacgacagcaatgtgaagaacctgtacgagaaggtgagaagccagctgaagaacaatgccaaggagatcggcaacggctgctttgagttctaccacaagtgtgacaacacctgtatggagtctgtgaagaacggcacctacgactaccctaagtatagcgaggaggccaagctgaatagagaggagatcgacggcgtgaaactggaaagcacaagaatctatcagggcgctgaaaacctgtattttcagggcggttctggttacatcccggaagctccgcgtgacggtcaggcttacgttcgtaaagacggtgaatgggttctgctgtctaccttcctgggtcaccatcatcaccaccatcaccatcatcactgataaaagctt

SEQ ID NO: 38 - protein, 588 aa, Artificial Sequence
  Synthetic
MVSAIVLYVLLAAAAHSAFADTLCIGYHANNSTDTVDTVLEKNVTVTHSVNLLEDKHNGKLCKLRGVAPLHLGKCNIAGWILGNPECESLSTASSWSYIVETPSSDNGTCYPGDFIDYEELREQLSSVSSFERFEIFPKTSSWPNHDSNKGVTAACPGIFGAIAGFIEGFYKNLIWLVKKGNSYPKLSKSYINDKGKEVLVLWGIHHPSTSADQQSLYQNADAYVFVGSSRYSKKFKPEIAIRPKVRDQEGRMNYYWTLVEPGDKITFEATGNLVVPRYAFAMERNAGSGIIISDTPVHDCNTTCQTPKGAINTSLPFQNIHPITIGKCPKYVKSTKLRLATGLRNSPENLYFQGLFGAIAGFIEGGWTGMVDGWYGYHHQNEQGSGYAADLKSTQNAIDEITNKVNSVIEKMNTQFTAVGKEFNHLEKRIENLNKKVDDGFLDIWTYNAELLVLLENERTLDYHDSNVKNLYEKVRSQLKNNAKEIGNGCFEFYHKCDNTCMESVKNGTYDYPKYSEEAKLNREEIDGVKLESTRIYQGAENLYFQGGSGYIPEAPRDGQAYVRKDGEWVLLSTFLGHHHHHHHHHH

SEQ ID NO: 39 - DNA, 1778 bp, Artificial Sequence
  Synthetic
ccatggtaagcgctattgttttatatgtgcttttggcggcggcggcgcattctgcctttgcggatacactgtgtattggctaccacgccaacaatagcaccgataccgtggatacagtgctggagaagaatgtgaccgtgacccactctgtgaatctgctggaggataagcacaatggcaagctgtgtaagctgagaggagttgcccctctgcacctgggcaaatgtaatattgccggctggattctgggaaatcctgaatgtgaaagcctgtctacagccagcagctggtcttatatcgtggaaacccctagcagcgacaatggcacctgttaccctggcgacttcatcgattacgaggagctgagagaacagctgtctagcgtgtccagcttcgagagattcgagatcttccctaagacaagcagctggcctaatcacgattctaataagggagtgacagccgcctgtcctggcattttcggcgctatcgccggcttcattgagggattttacaagaacctgatctggctggtgaagaagggcaacagctaccctaagctgtctaagagctacatcaacgacaagggcaaagaagtgctggtgctgtggggaatccaccaccctagcacaagcgccgatcagcagagcctgtaccagaatgccgatgcctatgtgtttgtgggcagcagcagatacagcaaaaagttcaagcctgaaattgccattagacccaaagtgagagatcaggaaggcagaatgaattactactggaccctggtggaacctggcgataagatcacatttgaggccaccggaaatctggtggtgcctagatatgcatttgctatggagagaaatgctggctctggcatcattatctctgatacccctgtgcacgactgtaataccacctgtcagacacctaagggcgccattaataccagcctgcccttccagaatattcaccctatcaccatcggcaagtgtcctaagtatgtgaagagcaccaagctgagactggctaccggtctgagaaatagccctgaaaacctgtattttcaaggcctgtttggagccatcgccggctttattgagggaggatggaccggaatggtggatggctggtacggctatcaccaccagaatgagcagggatccggatatgccgccgatctgaagtctacacagaacgccatcgacgagatcacaaacaaggtgaacagcgtgatcgagaagatgaacacccagtttacagctgtgggcaaggagttcaaccacctggagaagagaatcgagaacctgaacaagaaagtggacgacggcttcctggatatttggacctacaatgccgagctgctcgtgctcctggagaatgagagaaccctggactaccacgacagcaatgtgaagaacctgtacgagaaggtgagaagccagctgaagaacaatgccaaggagatcggcaacggctgctttgagttctaccacaagtgtgacaacacctgtatggagtctgtgaagaacggcacctacgactaccctaagtatagcgaggaggccaagctgaatagagaggagatcgacggcgtgaaactggaaagcacaagaatctatcagggcgctgaaaacctgtattttcagggcggttctggttacatcccggaagctccgcgtgacggtcaggcttacgttcgtaaagacggtgaatgggttctgctgtctaccttcctgggtcaccatcatcaccaccatcaccatcatcactgataaaagctt

SEQ ID NO: 40 - protein, 589 aa, Artificial Sequence
  Synthetic
MVSAIVLYVLLAAAAHSAFADTLCIGYHANNSTDTVDTVLEKNVTVTHSVNLLEDKHNGKLCKLRGVAPLHLGKCNIAGWILGNPECESLSTASSWSYIVETPSSDNGTCYPGDFIDYEELREQLSSVSSFERFEIFPKTSSWPNHDSNKGVTAACPHAGAKSFYKNLIWLVGIFGAIAGFIEGYPKLSKSYINDKGKEVLVLWGIHHPSTSADQQSLYQNADAYVFVGSSRYSKKFKPEIAIRPKVRDQEGRMNYYWTLVEPGDKITFEATGNLVVPRYAFAMERNAGSGIIISDTPVHDCNTTCQTPKGAINTSLPFQNIHPITIGKCPKYVKSTKLRLATGLRNSPENLYFQGLFGAIAGFIEGGWTGMVDGWYGYHHQNEQGSGYAADLKSTQNAIDEITNKVNSVIEKMNTQFTAVGKEFNHLEKRIENLNKKVDDGFLDIWTYNAELLVLLENERTLDYHDSNVKNLYEKVRSQLKNNAKEIGNGCFEFYHKCDNTCMESVKNGTYDYPKYSEEAKLNREEIDGVKLESTRIYQGAENLYFQGGSGYIPEAPRDGQAYVRKDGEWVLLSTFLGHHHHHHHHHH

SEQ ID NO: 41 - DNA, 1781 bp, Artificial Sequence
  Synthetic
ccatggtaagcgctattgttttatatgtgcttttggcggcggcggcgcattctgcctttgcggatacactgtgtattggctaccacgccaacaatagcaccgataccgtggatacagtgctggagaagaatgtgaccgtgacccactctgtgaatctgctggaggataagcacaatggcaagctgtgtaagctgagaggagttgcccctctgcacctgggcaaatgtaatattgccggctggattctgggaaatcctgaatgtgaaagcctgtctacagccagcagctggtcttatatcgtggaaacccctagcagcgacaatggcacctgttaccctggcgacttcatcgattacgaggagctgagagaacagctgtctagcgtgtccagcttcgagagattcgagatcttccctaagacaagcagctggcctaatcacgattctaataagggagtgacagccgcctgtcctcatgccggagccaagtccttttacaagaacctgatctggctggtgggcattttcggcgctatcgccggcttcattgagggataccctaagctgtctaagagctacatcaacgacaagggcaaagaagtgctggtgctgtggggaatccaccaccctagcacaagcgccgatcagcagagcctgtaccagaatgccgatgcctatgtgtttgtgggcagcagcagatacagcaaaaagttcaagcctgaaattgccattagacccaaagtgagagatcaggaaggcagaatgaattactactggaccctggtggaacctggcgataagatcacatttgaggccaccggaaatctggtggtgcctagatatgcatttgctatggagagaaatgctggctctggcatcattatctctgatacccctgtgcacgactgtaataccacctgtcagacacctaagggcgccattaataccagcctgcccttccagaatattcaccctatcaccatcggcaagtgtcctaagtatgtgaagagcaccaagctgagactggctaccggtctgagaaatagccctgaaaacctgtattttcaaggcctgtttggagccatcgccggctttattgagggaggatggaccggaatggtggatggctggtacggctatcaccaccagaatgagcagggatccggatatgccgccgatctgaagtctacacagaacgccatcgacgagatcacaaacaaggtgaacagcgtgatcgagaagatgaacacccagtttacagctgtgggcaaggagttcaaccacctggagaagagaatcgagaacctgaacaagaaagtggacgacggcttcctggatatttggacctacaatgccgagctgctcgtgctcctggagaatgagagaaccctggactaccacgacagcaatgtgaagaacctgtacgagaaggtgagaagccagctgaagaacaatgccaaggagatcggcaacggctgctttgagttctaccacaagtgtgacaacacctgtatggagtctgtgaagaacggcacctacgactaccctaagtatagcgaggaggccaagctgaatagagaggagatcgacggcgtgaaactggaaagcacaagaatctatcagggcgctgaaaacctgtattttcagggcggttctggttacatcccggaagctccgcgtgacggtcaggcttacgttcgtaaagacggtgaatgggttctgctgtctaccttcctgggtcaccatcatcaccaccatcaccatcatcactgataaaagctt

SEQ ID NO: 42 - protein, 590 aa, Artificial Sequence
  Synthetic
MVSAIVLYVLLAAAAHSAFADTLCIGYHANNSTDTVDTVLEKNVTVTHSVNLLEDKHNGKLCKLRGVAPLHLGKCNIAGWILGNPECESLSTASSWSYIVETPSSDNGTCYPGDFIDYEELREQLSSVSSFERFEIFPGIFGAIAGFIEGWPNHDSNKGVTAACPHAGAKSFYKNLIWLVKKGNSYPKLSKSYINDKGKEVLVLWGIHHPSTSADQQSLYQNADAYVFVGSSRYSKKFKPEIAIRPKVRDQEGRMNYYWTLVEPGDKITFEATGNLVVPRYAFAMERNAGSGIIISDTPVHDCNTTCQTPKGAINTSLPFQNIHPITIGKCPKYVKSTKLRLATGLRNSPENLYFQGLFGAIAGFIEGGWTGMVDGWYGYHHQNEQGSGYAADLKSTQNAIDEITNKVNSVIEKMNTQFTAVGKEFNHLEKRIENLNKKVDDGFLDIWTYNAELLVLLENERTLDYHDSNVKNLYEKVRSQLKNNAKEIGNGCFEFYHKCDNTCMESVKNGTYDYPKYSEEAKLNREEIDGVKLESTRIYQGAENLYFQGGSGYIPEAPRDGQAYVRKDGEWVLLSTFLGHHHHHHHHHH

SEQ ID NO: 43 - DNA, 1784 bp, Artificial Sequence
  Synthetic
ccatggtaagcgctattgttttatatgtgcttttggcggcggcggcgcattctgcctttgcggatacactgtgtattggctaccacgccaacaatagcaccgataccgtggatacagtgctggagaagaatgtgaccgtgacccactctgtgaatctgctggaggataagcacaatggcaagctgtgtaagctgagaggagttgcccctctgcacctgggcaaatgtaatattgccggctggattctgggaaatcctgaatgtgaaagcctgtctacagccagcagctggtcttatatcgtggaaacccctagcagcgacaatggcacctgttaccctggcgacttcatcgattacgaggagctgagagaacagctgtctagcgtgtccagcttcgagagattcgagatcttccctggcattttcggcgctatcgccggcttcattgagggatggcctaatcacgattctaataagggagtgacagccgcctgtcctcatgccggagccaagtccttttacaagaacctgatctggctggtgaagaagggcaacagctaccctaagctgtctaagagctacatcaacgacaagggcaaagaagtgctggtgctgtggggaatccaccaccctagcacaagcgccgatcagcagagcctgtaccagaatgccgatgcctatgtgtttgtgggcagcagcagatacagcaaaaagttcaagcctgaaattgccattagacccaaagtgagagatcaggaaggcagaatgaattactactggaccctggtggaacctggcgataagatcacatttgaggccaccggaaatctggtggtgcctagatatgcatttgctatggagagaaatgctggctctggcatcattatctctgatacccctgtgcacgactgtaataccacctgtcagacacctaagggcgccattaataccagcctgcccttccagaatattcaccctatcaccatcggcaagtgtcctaagtatgtgaagagcaccaagctgagactggctaccggtctgagaaatagccctgaaaacctgtattttcaaggcctgtttggagccatcgccggctttattgagggaggatggaccggaatggtggatggctggtacggctatcaccaccagaatgagcagggatccggatatgccgccgatctgaagtctacacagaacgccatcgacgagatcacaaacaaggtgaacagcgtgatcgagaagatgaacacccagtttacagctgtgggcaaggagttcaaccacctggagaagagaatcgagaacctgaacaagaaagtggacgacggcttcctggatatttggacctacaatgccgagctgctcgtgctcctggagaatgagagaaccctggactaccacgacagcaatgtgaagaacctgtacgagaaggtgagaagccagctgaagaacaatgccaaggagatcggcaacggctgctttgagttctaccacaagtgtgacaacacctgtatggagtctgtgaagaacggcacctacgactaccctaagtatagcgaggaggccaagctgaatagagaggagatcgacggcgtgaaactggaaagcacaagaatctatcagggcgctgaaaacctgtattttcagggcggttctggttacatcccggaagctccgcgtgacggtcaggcttacgttcgtaaagacggtgaatgggttctgctgtctaccttcctgggtcaccatcatcaccaccatcaccatcatcactgataaaagctt

SEQ ID NO: 44 - protein, 584 aa, Artificial Sequence
  Synthetic
MVSAIVLYVLLAAAAHSAFADTLCIGYHANNSTDTVDTVLEKNVTVTHSVNLLEDKHNGKLCKLRGVAPLHLGKCNIAGWILGNPECESLSTASSWSYIVETPSSDNGTCYPGDFIDYEELREQLSSVSSFERFEIFPKTSSWPNHDSNKGVTAACPHAGAKSFYKNLIWLVKKGNSYPKLSKSYINDKGKEVLVLWGIHHPSGIFGAIAGFIEGDAYVFVGSSRYSKKFKPEIAIRPKVRDQEGRMNYYWTLVEPGDKITFEATGNLVVPRYAFAMERNAGSGIIISDTPVHDCNTTCQTPKGAINTSLPFQNIHPITIGKCPKYVKSTKLRLATGLRNSPQRERRKKRGLFGAIAGFIEGGWTGMVDGWYGYHHQNEQGSGYAADLKSTQNAIDEITNKVNSVIEKMNTQFTAVGKEFNHLEKRIENLNKKVDDGFLDIWTYNAELLVLLENERTLDYHDSNVKNLYEKVRSQLKNNAKEIGNGCFEFYHKCDNTCMESVKNGTYDYPKYSEEAKLNREEIDGVKLESTRIYQGAENLYFQGGSGYIPEAPRDGQAYVRKDGEWVLLSTFLGHHHHHHHHHH

SEQ ID NO: 45 - DNA, 1766 bp, Artificial Sequence
  Synthetic
ccatggtaagcgctattgttttatatgtgcttttggcggcggcggcgcattctgcctttgcggatacactgtgtattggctaccacgccaacaatagcaccgataccgtggatacagtgctggagaagaatgtgaccgtgacccactctgtgaatctgctggaggataagcacaatggcaagctgtgtaagctgagaggagttgcccctctgcacctgggcaaatgtaatattgccggctggattctgggaaatcctgaatgtgaaagcctgtctacagccagcagctggtcttatatcgtggaaacccctagcagcgacaatggcacctgttaccctggcgacttcatcgattacgaggagctgagagaacagctgtctagcgtgtccagcttcgagagattcgagatcttccctaagacaagcagctggcctaatcacgattctaataagggagtgacagccgcctgtcctcatgccggagccaagtccttttacaagaacctgatctggctggtgaagaagggcaacagctaccctaagctgtctaagagctacatcaacgacaagggcaaagaagtgctggtgctgtggggaatccaccaccctagcggcattttcggcgctatcgccggcttcattgagggagatgcctatgtgtttgtgggcagcagcagatacagcaaaaagttcaagcctgaaattgccattagacccaaagtgagagatcaggaaggcagaatgaattactactggaccctggtggaacctggcgataagatcacatttgaggccaccggaaatctggtggtgcctagatatgcatttgctatggagagaaatgctggctctggcatcattatctctgatacccctgtgcacgactgtaataccacctgtcagacacctaagggcgccattaataccagcctgcccttccagaatattcaccctatcaccatcggcaagtgtcctaagtatgtgaagagcaccaagctgagactggctaccggtctgagaaatagccctcagagggagagacgcaagaagagaggcctgtttggagccatcgccggctttattgagggaggatggaccggaatggtggatggctggtacggctatcaccaccagaatgagcagggatccggatatgccgccgatctgaagtctacacagaacgccatcgacgagatcacaaacaaggtgaacagcgtgatcgagaagatgaacacccagtttacagctgtgggcaaggagttcaaccacctggagaagagaatcgagaacctgaacaagaaagtggacgacggcttcctggatatttggacctacaatgccgagctgctcgtgctcctggagaatgagagaaccctggactaccacgacagcaatgtgaagaacctgtacgagaaggtgagaagccagctgaagaacaatgccaaggagatcggcaacggctgctttgagttctaccacaagtgtgacaacacctgtatggagtctgtgaagaacggcacctacgactaccctaagtatagcgaggaggccaagctgaatagagaggagatcgacggcgtgaaactggaaagcacaagaatctatcagggcgctgaaaacctgtattttcagggcggttctggttacatcccggaagctccgcgtgacggtcaggcttacgttcgtaaagacggtgaatgggttctgctgtctaccttcctgggtcaccatcatcaccaccatcaccatcatcactgataaaagctt

SEQ ID NO: 46 - protein, 584 aa, Artificial Sequence
  Synthetic
MVSAIVLYVLLAAAAHSAFADTLCIGYHANNSTDTVDTVLEKNVTVTHSVNLLEDKHNGKLCKLRGVAPLHLGKCNIAGWILGNPECESLSTASSWSYIVETPSSDNGTCYPGDFIDYEELREQLSSVSSFERFEIFPKTSSWPNHDSNKGVTAACPHAGAKSFYKNLIWLVKKGNSYPKLSKSYINDKGKEVLVLWGIHHPSTSADQQSLYQNADAYVFVGSSRYSKKFKPGIFGAIAGFIEGGRMNYYWTLVEPGDKITFEATGNLVVPRYAFAMERNAGSGIIISDTPVHDCNTTCQTPKGAINTSLPFQNIHPITIGKCPKYVKSTKLRLATGLRNSPQRERRKKRGLFGAIAGFIEGGWTGMVDGWYGYHHQNEQGSGYAADLKSTQNAIDEITNKVNSVIEKMNTQFTAVGKEFNHLEKRIENLNKKVDDGFLDIWTYNAELLVLLENERTLDYHDSNVKNLYEKVRSQLKNNAKEIGNGCFEFYHKCDNTCMESVKNGTYDYPKYSEEAKLNREEIDGVKLESTRIYQGAENLYFQGGSGYIPEAPRDGQAYVRKDGEWVLLSTFLGHHHHHHHHHH

SEQ ID NO: 47 - DNA, 1766 bp, Artificial Sequence
  Synthetic
ccatggtaagcgctattgttttatatgtgcttttggcggcggcggcgcattctgcctttgcggatacactgtgtattggctaccacgccaacaatagcaccgataccgtggatacagtgctggagaagaatgtgaccgtgacccactctgtgaatctgctggaggataagcacaatggcaagctgtgtaagctgagaggagttgcccctctgcacctgggcaaatgtaatattgccggctggattctgggaaatcctgaatgtgaaagcctgtctacagccagcagctggtcttatatcgtggaaacccctagcagcgacaatggcacctgttaccctggcgacttcatcgattacgaggagctgagagaacagctgtctagcgtgtccagcttcgagagattcgagatcttccctaagacaagcagctggcctaatcacgattctaataagggagtgacagccgcctgtcctcatgccggagccaagtccttttacaagaacctgatctggctggtgaagaagggcaacagctaccctaagctgtctaagagctacatcaacgacaagggcaaagaagtgctggtgctgtggggaatccaccaccctagcacaagcgccgatcagcagagcctgtaccagaatgccgatgcctatgtgtttgtgggcagcagcagatacagcaaaaagttcaagcctggcattttcggcgctatcgccggcttcattgagggaggcagaatgaattactactggaccctggtggaacctggcgataagatcacatttgaggccaccggaaatctggtggtgcctagatatgcatttgctatggagagaaatgctggctctggcatcattatctctgatacccctgtgcacgactgtaataccacctgtcagacacctaagggcgccattaataccagcctgcccttccagaatattcaccctatcaccatcggcaagtgtcctaagtatgtgaagagcaccaagctgagactggctaccggtctgagaaatagccctcagagggagagacgcaagaagagaggcctgtttggagccatcgccggctttattgagggaggatggaccggaatggtggatggctggtacggctatcaccaccagaatgagcagggatccggatatgccgccgatctgaagtctacacagaacgccatcgacgagatcacaaacaaggtgaacagcgtgatcgagaagatgaacacccagtttacagctgtgggcaaggagttcaaccacctggagaagagaatcgagaacctgaacaagaaagtggacgacggcttcctggatatttggacctacaatgccgagctgctcgtgctcctggagaatgagagaaccctggactaccacgacagcaatgtgaagaacctgtacgagaaggtgagaagccagctgaagaacaatgccaaggagatcggcaacggctgctttgagttctaccacaagtgtgacaacacctgtatggagtctgtgaagaacggcacctacgactaccctaagtatagcgaggaggccaagctgaatagagaggagatcgacggcgtgaaactggaaagcacaagaatctatcagggcgctgaaaacctgtattttcagggcggttctggttacatcccggaagctccgcgtgacggtcaggcttacgttcgtaaagacggtgaatgggttctgctgtctaccttcctgggtcaccatcatcaccaccatcaccatcatcactgataaaagctt

SEQ ID NO: 48 - protein, 592 aa, Artificial Sequence
  Synthetic
MVSAIVLYVLLAAAAHSAFADTLCIGYHANNSTDTVDTVLEKNVTVTHSVNLLEDKHNGKLCKLRGVAPLHLGKCNIAGWILGNPECESLSTASSWSYIVETPSSDNGTCYPGDFIDYEELREQLSSVSSFERFEIFPKTSSWPNHDSNKGVTAACPHAGAKSFYKNLIWLVRKKRGLFGAIAGFIEYINDKGKEVLVLWGIHHPSKESTQKAIDGVTNKVNSDAYVFVGSSRYSKKFKPEIAIRPKVRDQEGRMNYYWTLVEPGDKITFEATGNLVVPRYAFAMERNAGSGIIISDTPVHDCNTTCQTPKGAINTSLPFQNIHPITIGKCPKYVKSTKLRLATGLRNSPQRERRKKRGLFGAIAGFIEGGWTGMVDGWYGYHHQNEQGSGYAADLKSTQNAIDEITNKVNSVIEKMNTQFTAVGKEFNHLEKRIENLNKKVDDGFLDIWTYNAELLVLLENERTLDYHDSNVKNLYEKVRSQLKNNAKEIGNGCFEFYHKCDNTCMESVKNGTYDYPKYSEEAKLNREEIDGVKLESTRIYQGAENLYFQGGSGYIPEAPRDGQAYVRKDGEWVLLSTFLGHHHHHHHHHH

SEQ ID NO: 49 - protein, 15 aa, Artificial Sequence
  Synthetic
RKKRGLFGAIAGFIE

SEQ ID NO: 50 - protein, 17 aa, Artificial Sequence
  Synthetic
KESTQKAIDGVTNKVNS

SEQ ID NO: 51 - DNA, 1790 bp, Artificial Sequence
  Synthetic
ccatggtaagcgctattgttttatatgtgcttttggcggcggcggcgcattctgcctttgcggatacactgtgtattggctaccacgccaacaatagcaccgataccgtggatacagtgctggagaagaatgtgaccgtgacccactctgtgaatctgctggaggataagcacaatggcaagctgtgtaagctgagaggagttgcccctctgcacctgggcaaatgtaatattgccggctggattctgggaaatcctgaatgtgaaagcctgtctacagccagcagctggtcttatatcgtggaaacccctagcagcgacaatggcacctgttaccctggcgacttcatcgattacgaggagctgagagaacagctgtctagcgtgtccagcttcgagagattcgagatcttccctaagacaagcagctggcctaatcacgattctaataagggagtgacagccgcctgtcctcatgccggagccaagtccttttacaagaacctgatctggctggtgagaaagaagagaggcctgtttggagccatcgccggctttattgagtacatcaacgacaagggcaaagaagtgctggtgctgtggggaatccaccaccctagcaaggagtctacacagaaggccattgatggcgttacaaataaggtcaattctgatgcctatgtgtttgtgggcagcagcagatacagcaaaaagttcaagcctgaaattgccattagacccaaagtgagagatcaggaaggcagaatgaattactactggaccctggtggaacctggcgataagatcacatttgaggccaccggaaatctggtggtgcctagatatgcatttgctatggagagaaatgctggctctggcatcattatctctgatacccctgtgcacgactgtaataccacctgtcagacacctaagggcgccattaataccagcctgcccttccagaatattcaccctatcaccatcggcaagtgtcctaagtatgtgaagagcaccaagctgagactggctaccggtctgagaaatagccctcagagggagagacgcaagaagagaggcctgtttggagccatcgccggctttattgagggaggatggaccggaatggtggatggctggtacggctatcaccaccagaatgagcagggatccggatatgccgccgatctgaagtctacacagaacgccatcgacgagatcacaaacaaggtgaacagcgtgatcgagaagatgaacacccagtttacagctgtgggcaaggagttcaaccacctggagaagagaatcgagaacctgaacaagaaagtggacgacggcttcctggatatttggacctacaatgccgagctgctcgtgctcctggagaatgagagaaccctggactaccacgacagcaatgtgaagaacctgtacgagaaggtgagaagccagctgaagaacaatgccaaggagatcggcaacggctgctttgagttctaccacaagtgtgacaacacctgtatggagtctgtgaagaacggcacctacgactaccctaagtatagcgaggaggccaagctgaatagagaggagatcgacggcgtgaaactggaaagcacaagaatctatcagggcgctgaaaacctgtattttcagggcggttctggttacatcccggaagctccgcgtgacggtcaggcttacgttcgtaaagacggtgaatgggttctgctgtctaccttcctgggtcaccatcatcaccaccatcaccatcatcactgataaaagctt

SEQ ID NO: 52 - protein, 589 aa, Artificial Sequence
  Synthetic
MVSAIVLYVLLAAAAHSAFADTLCIGYHANNSTDTVDTVLEKNVTVTHSVNLLEDKHNGKLCKLRGVAPLHLGKCNIAGWILGNPECESLSTASSWSYIVETPSSDNGTCYPGDFIDYEELREQLSSVSSFERFEIFPKTSSWPNHDSNKGVTAACPHAGAKSFYKNLIWLVRKKRGLFGAIAGFIEYINDKGKEVLVLWGIHHPSKESTQKAIDGVTNKVNSDAYVFVGSSRYSKKFKPEIAIRPKVRDQEGRMNYYWTLVEPGDKITFEATGNLVVPRYAFAMERNAGSGIIISDTPVHDCNTTCQTPKGAINTSLPFQNIHPITIGKCPKYVKSTKLRLATGLRNIPSIQSRGLFGAIAGFIEGGWTGMVDGWYGYHHQNEQGSGYAADLKSTQNAIDEITNKVNSVIEKMNTQFTAVGKEFNHLEKRIENLNKKVDDGFLDIWTYNAELLVLLENERTLDYHDSNVKNLYEKVRSQLKNNAKEIGNGCFEFYHKCDNTCMESVKNGTYDYPKYSEEAKLNREEIDGVKLESTRIYQGAENLYFQGGSGYIPEAPRDGQAYVRKDGEWVLLSTFLGHHHHHHHHHH

SEQ ID NO: 53 - DNA, 1781 bp, Artificial Sequence
  Synthetic
ccatggtaagcgctattgttttatatgtgcttttggcggcggcggcgcattctgcctttgcggatacactgtgtattggctaccacgccaacaatagcaccgataccgtggatacagtgctggagaagaatgtgaccgtgacccactctgtgaatctgctggaggataagcacaatggcaagctgtgtaagctgagaggagttgcccctctgcacctgggcaaatgtaatattgccggctggattctgggaaatcctgaatgtgaaagcctgtctacagccagcagctggtcttatatcgtggaaacccctagcagcgacaatggcacctgttaccctggcgacttcatcgattacgaggagctgagagaacagctgtctagcgtgtccagcttcgagagattcgagatcttccctaagacaagcagctggcctaatcacgattctaataagggagtgacagccgcctgtcctcatgccggagccaagtccttttacaagaacctgatctggctggtgagaaagaagagaggcctgtttggagccatcgccggctttattgagtacatcaacgacaagggcaaagaagtgctggtgctgtggggaatccaccaccctagcaaggagtctacacagaaggccattgatggcgttacaaataaggtcaattctgatgcctatgtgtttgtgggcagcagcagatacagcaaaaagttcaagcctgaaattgccattagacccaaagtgagagatcaggaaggcagaatgaattactactggaccctggtggaacctggcgataagatcacatttgaggccaccggaaatctggtggtgcctagatatgcatttgctatggagagaaatgctggctctggcatcattatctctgatacccctgtgcacgactgtaataccacctgtcagacacctaagggcgccattaataccagcctgcccttccagaatattcaccctatcaccatcggcaagtgtcctaagtatgtgaagagcaccaagctgagactggctaccggtctgagaaatatccctagcatccagagcagaggcctgtttggagccatcgccggctttattgagggaggatggaccggaatggtggatggctggtacggctatcaccaccagaatgagcagggatccggatatgccgccgatctgaagtctacacagaacgccatcgacgagatcacaaacaaggtgaacagcgtgatcgagaagatgaacacccagtttacagctgtgggcaaggagttcaaccacctggagaagagaatcgagaacctgaacaagaaagtggacgacggcttcctggatatttggacctacaatgccgagctgctcgtgctcctggagaatgagagaaccctggactaccacgacagcaatgtgaagaacctgtacgagaaggtgagaagccagctgaagaacaatgccaaggagatcggcaacggctgctttgagttctaccacaagtgtgacaacacctgtatggagtctgtgaagaacggcacctacgactaccctaagtatagcgaggaggccaagctgaatagagaggagatcgacggcgtgaaactggaaagcacaagaatctatcagggcgctgaaaacctgtattttcagggcggttctggttacatcccggaagctccgcgtgacggtcaggcttacgttcgtaaagacggtgaatgggttctgctgtctaccttcctgggtcaccatcatcaccaccatcaccatcatcactgataaaagctt

SEQ ID NO: 54 - protein, 585 aa, Artificial Sequence
  Synthetic
MVSAIVLYVLLAAAAHSAFADTLCIGYHANNSTDTVDTVLEKNVTVTHSVNLLEDKHNGKLCKLRGVAPLHLGKCNIAGWILGNPECESLSTASSWSYIVETPSSDNGTCYPGDFIDYEELREQLSSVSSFERFEIFPKTSSWPNHDSNKGVTAACPHAGAKSFYKNLIWLVRKKRGLFGAIAGFIEGYINDKGKEVLVLWGIHHPSTSADQQSLYQNADAYVFVGSSRYSKKFKPEIAIRPKVRDQEGRMNYYWTLVEPGDKITFEATGNLVVPRYAFAMERNAGSGIIISDTPVHDCNTTCQTPKGAINTSLPFQNIHPITIGKCPKYVKSTKLRLATGLRNIENLYFQGLFGAIAGFIEGGWTGMVDGWYGYHHQNEQGSGYAADLKSTQNAIDEITNKVNSVIEKMNTQFTAVGKEFNHLEKRIENLNKKVDDGFLDIWTYNAELLVLLENERTLDYHDSNVKNLYEKVRSQLKNNAKEIGNGCFEFYHKCDNTCMESVKNGTYDYPKYSEEAKLNREEIDGVKLESTRIYQGAENLYFQGGSGYIPEAPRDGQAYVRKDGEWVLLSTFLGHHHHHHHHHH

SEQ ID NO: 55 - DNA, 1769 bp, Artificial Sequence
  Synthetic
ccatggtaagcgctattgttttatatgtgcttttggcggcggcggcgcattctgcctttgcggatacactgtgtattggctaccacgccaacaatagcaccgataccgtggatacagtgctggagaagaatgtgaccgtgacccactctgtgaatctgctggaggataagcacaatggcaagctgtgtaagctgagaggagttgcccctctgcacctgggcaaatgtaatattgccggctggattctgggaaatcctgaatgtgaaagcctgtctacagccagcagctggtcttatatcgtggaaacccctagcagcgacaatggcacctgttaccctggcgacttcatcgattacgaggagctgagagaacagctgtctagcgtgtccagcttcgagagattcgagatcttccctaagacaagcagctggcctaatcacgattctaataagggagtgacagccgcctgtcctcatgccggagccaagtccttttacaagaacctgatctggctggtgagaaagaagagaggcctgttcggcgctatcgccggcttcattgagggatacatcaacgacaagggcaaagaagtgctggtgctgtggggaatccaccaccctagcacaagcgccgatcagcagagcctgtaccagaatgccgatgcctatgtgtttgtgggcagcagcagatacagcaaaaagttcaagcctgaaattgccattagacccaaagtgagagatcaggaaggcagaatgaattactactggaccctggtggaacctggcgataagatcacatttgaggccaccggaaatctggtggtgcctagatatgcatttgctatggagagaaatgctggctctggcatcattatctctgatacccctgtgcacgactgtaataccacctgtcagacacctaagggcgccattaataccagcctgcccttccagaatattcaccctatcaccatcggcaagtgtcctaagtatgtgaagagcaccaagctgagactggctaccggtctgagaaatatcgaaaacctgtattttcaaggcctgtttggagccatcgccggctttattgagggaggatggaccggaatggtggatggctggtacggctatcaccaccagaatgagcagggatccggatatgccgccgatctgaagtctacacagaacgccatcgacgagatcacaaacaaggtgaacagcgtgatcgagaagatgaacacccagtttacagctgtgggcaaggagttcaaccacctggagaagagaatcgagaacctgaacaagaaagtggacgacggcttcctggatatttggacctacaatgccgagctgctcgtgctcctggagaatgagagaaccctggactaccacgacagcaatgtgaagaacctgtacgagaaggtgagaagccagctgaagaacaatgccaaggagatcggcaacggctgctttgagttctaccacaagtgtgacaacacctgtatggagtctgtgaagaacggcacctacgactaccctaagtatagcgaggaggccaagctgaatagagaggagatcgacggcgtgaaactggaaagcacaagaatctatcagggcgctgaaaacctgtattttcagggcggttctggttacatcccggaagctccgcgtgacggtcaggcttacgttcgtaaagacggtgaatgggttctgctgtctaccttcctgggtcaccatcatcaccaccatcaccatcatcactgataaaagctt

SEQ ID NO: 56 - protein, 593 aa, Artificial Sequence
  Synthetic
MVSAIVLYVLLAAAAHSAFADTLCIGYHANNSTDTVDTVLEKNVTVTHSVNLLEDKHNGKLCKLRGVAPLHLGKCNIAGWILGNPECESLSTASSWSYIVETPSSDNGTCYPGDFIDYEELREQLSSVSSFERFEIFPKTSSWPNHDSNKGVTAACPHAGAKSFYKNLIWLVKKGNSYPKLSKSYINDKGKEVLVLWGIHHPSTSADQQSLYQNADAYVFVGSSRYSKKFKPSLLTEVETPTRNGWECKCSDSGRMNYYWTLVEPGDKITFEATGNLVVPRYAFAMERNAGSGIIISDTPVHDCNTTCQTPKGAINTSLPFQNIHPITIGKCPKYVKSTKLRLATGLRNSPQRERRKKRGLFGAIAGFIEGGWTGMVDGWYGYHHQNEQGSGYAADLKSTQNAIDEITNKVNSVIEKMNTQFTAVGKEFNHLEKRIENLNKKVDDGFLDIWTYNAELLVLLENERTLDYHDSNVKNLYEKVRSQLKNNAKEIGNGCFEFYHKCDNTCMESVKNGTYDYPKYSEEAKLNREEIDGVKLESTRIYQGAENLYFQGGSGYIPEAPRDGQAYVRKDGEWVLLSTFLGHHHHHHHHHH

SEQ ID NO: 57 - protein, 21 aa, Artificial Sequence
  Synthetic
SLLTEVETPTRNGWECKCSDS

SEQ ID NO: 58 - DNA, 1793 bp, Artificial Sequence
  Synthetic
ccatggtaagcgctattgttttatatgtgcttttggcggcggcggcgcattctgcctttgcggatacactgtgtattggctaccacgccaacaatagcaccgataccgtggatacagtgctggagaagaatgtgaccgtgacccactctgtgaatctgctggaggataagcacaatggcaagctgtgtaagctgagaggagttgcccctctgcacctgggcaaatgtaatattgccggctggattctgggaaatcctgaatgtgaaagcctgtctacagccagcagctggtcttatatcgtggaaacccctagcagcgacaatggcacctgttaccctggcgacttcatcgattacgaggagctgagagaacagctgtctagcgtgtccagcttcgagagattcgagatcttccctaagacaagcagctggcctaatcacgattctaataagggagtgacagccgcctgtcctcatgccggagccaagtccttttacaagaacctgatctggctggtgaagaagggcaacagctaccctaagctgtctaagagctacatcaacgacaagggcaaagaagtgctggtgctgtggggaatccaccaccctagcacaagcgccgatcagcagagcctgtaccagaatgccgatgcctatgtgtttgtgggcagcagcagatacagcaaaaagttcaagccttccctgctgaccgaggtggagacccccaccaggaacggctgggagtgcaagtgctccgactccggcagaatgaattactactggaccctggtggaacctggcgataagatcacatttgaggccaccggaaatctggtggtgcctagatatgcatttgctatggagagaaatgctggctctggcatcattatctctgatacccctgtgcacgactgtaataccacctgtcagacacctaagggcgccattaataccagcctgcccttccagaatattcaccctatcaccatcggcaagtgtcctaagtatgtgaagagcaccaagctgagactggctaccggtctgagaaatagccctcagagggagagacgcaagaagagaggcctgtttggagccatcgccggctttattgagggaggatggaccggaatggtggatggctggtacggctatcaccaccagaatgagcagggatccggatatgccgccgatctgaagtctacacagaacgccatcgacgagatcacaaacaaggtgaacagcgtgatcgagaagatgaacacccagtttacagctgtgggcaaggagttcaaccacctggagaagagaatcgagaacctgaacaagaaagtggacgacggcttcctggatatttggacctacaatgccgagctgctcgtgctcctggagaatgagagaaccctggactaccacgacagcaatgtgaagaacctgtacgagaaggtgagaagccagctgaagaacaatgccaaggagatcggcaacggctgctttgagttctaccacaagtgtgacaacacctgtatggagtctgtgaagaacggcacctacgactaccctaagtatagcgaggaggccaagctgaatagagaggagatcgacggcgtgaaactggaaagcacaagaatctatcagggcgctgaaaacctgtattttcagggcggttctggttacatcccggaagctccgcgtgacggtcaggcttacgttcgtaaagacggtgaatgggttctgctgtctaccttcctgggtcaccatcatcaccaccatcaccatcatcactgataaaagctt

SEQ ID NO: 59 - protein, 593 aa, Artificial Sequence
  Synthetic
MVSAIVLYVLLAAAAHSAFADTLCIGYHANNSTDTVDTVLEKNVTVTHSVNLLEDKHNGKLCKLRGVAPLHLGKCNIAGWILGNPECESLSTASSWSYIVETPSSDNGTCYPGDFIDYEELREQLSSVSSFERFEIFPKTSSWPNHDSNKGVTAACPHAGAKSFYKNLIWLVKKGNSYPKLSKSYINDKGKEVLVLWGIHHPSSLLTEVETPTRNGWECKCSDSDAYVFVGSSRYSKKFKPEIAIRPKVRDQEGRMNYYWTLVEPGDKITFEATGNLVVPRYAFAMERNAGSGIIISDTPVHDCNTTCQTPKGAINTSLPFQNIHPITIGKCPKYVKSTKLRLATGLRNSPQRERRKKRGLFGAIAGFIEGGWTGMVDGWYGYHHQNEQGSGYAADLKSTQNAIDEITNKVNSVIEKMNTQFTAVGKEFNHLEKRIENLNKKVDDGFLDIWTYNAELLVLLENERTLDYHDSNVKNLYEKVRSQLKNNAKEIGNGCFEFYHKCDNTCMESVKNGTYDYPKYSEEAKLNREEIDGVKLESTRIYQGAENLYFQGGSGYIPEAPRDGQAYVRKDGEWVLLSTFLGHHHHHHHHHH

SEQ ID NO: 60 - DNA, 1793 bp, Artificial Sequence
  Synthetic
ccatggtaagcgctattgttttatatgtgcttttggcggcggcggcgcattctgcctttgcggatacactgtgtattggctaccacgccaacaatagcaccgataccgtggatacagtgctggagaagaatgtgaccgtgacccactctgtgaatctgctggaggataagcacaatggcaagctgtgtaagctgagaggagttgcccctctgcacctgggcaaatgtaatattgccggctggattctgggaaatcctgaatgtgaaagcctgtctacagccagcagctggtcttatatcgtggaaacccctagcagcgacaatggcacctgttaccctggcgacttcatcgattacgaggagctgagagaacagctgtctagcgtgtccagcttcgagagattcgagatcttccctaagacaagcagctggcctaatcacgattctaataagggagtgacagccgcctgtcctcatgccggagccaagtccttttacaagaacctgatctggctggtgaagaagggcaacagctaccctaagctgtctaagagctacatcaacgacaagggcaaagaagtgctggtgctgtggggaatccaccaccctagctccctgctgaccgaggtggagacccccaccaggaacggctgggagtgcaagtgctccgactccgatgcctatgtgtttgtgggcagcagcagatacagcaaaaagttcaagcctgaaattgccattagacccaaagtgagagatcaggaaggcagaatgaattactactggaccctggtggaacctggcgataagatcacatttgaggccaccggaaatctggtggtgcctagatatgcatttgctatggagagaaatgctggctctggcatcattatctctgatacccctgtgcacgactgtaataccacctgtcagacacctaagggcgccattaataccagcctgcccttccagaatattcaccctatcaccatcggcaagtgtcctaagtatgtgaagagcaccaagctgagactggctaccggtctgagaaatagccctcagagggagagacgcaagaagagaggcctgtttggagccatcgccggctttattgagggaggatggaccggaatggtggatggctggtacggctatcaccaccagaatgagcagggatccggatatgccgccgatctgaagtctacacagaacgccatcgacgagatcacaaacaaggtgaacagcgtgatcgagaagatgaacacccagtttacagctgtgggcaaggagttcaaccacctggagaagagaatcgagaacctgaacaagaaagtggacgacggcttcctggatatttggacctacaatgccgagctgctcgtgctcctggagaatgagagaaccctggactaccacgacagcaatgtgaagaacctgtacgagaaggtgagaagccagctgaagaacaatgccaaggagatcggcaacggctgctttgagttctaccacaagtgtgacaacacctgtatggagtctgtgaagaacggcacctacgactaccctaagtatagcgaggaggccaagctgaatagagaggagatcgacggcgtgaaactggaaagcacaagaatctatcagggcgctgaaaacctgtattttcagggcggttctggttacatcccggaagctccgcgtgacggtcaggcttacgttcgtaaagacggtgaatgggttctgctgtctaccttcctgggtcaccatcatcaccaccatcaccatcatcactgataaaagctt

SEQ ID NO: 61 - protein, 591 aa, Artificial Sequence
  Synthetic
MVSAIVLYVLLAAAAHSAFADTLCIGYHANNSTDTVDTVLEKNVTVTHSVNLLEDKHNGKLCKLRGVAPLHLGKCNIAGWILGNPECESLSTASSWSYIVETPSSDNGTCYPGDFIDYEELREQLSSVSSFERFEIFPKTSSWPNHDSNKGVTAACPHAGAKSFYKNLIWLVKKGNSYPKLSKSYINDKGKEVLVLWGIHHPSTSADQQSLYQNADAYVFVGSSRYSKKFKPSLLTEVETPTRNGWECKCSDSGRMNYYWTLVEPGDKITFEATGNLVVPRYAFAMERNAGSGIIISDTPVHDCNTTCQTPKGAINTSLPFQNIHPITIGKCPKYVKSTKLRLATGLRNSPENLYFQGLFGAIAGFIEGGWTGMVDGWYGYHHQNEQGSGYAADLKSTQNAIDEITNKVNSVIEKMNTQFTAVGKEFNHLEKRIENLNKKVDDGFLDIWTYNAELLVLLENERTLDYHDSNVKNLYEKVRSQLKNNAKEIGNGCFEFYHKCDNTCMESVKNGTYDYPKYSEEAKLNREEIDGVKLESTRIYQGAENLYFQGGSGYIPEAPRDGQAYVRKDGEWVLLSTFLGHHHHHHHHHH

SEQ ID NO: 62 - DNA, 1787 bp, Artificial Sequence
  Synthetic
ccatggtaagcgctattgttttatatgtgcttttggcggcggcggcgcattctgcctttgcggatacactgtgtattggctaccacgccaacaatagcaccgataccgtggatacagtgctggagaagaatgtgaccgtgacccactctgtgaatctgctggaggataagcacaatggcaagctgtgtaagctgagaggagttgcccctctgcacctgggcaaatgtaatattgccggctggattctgggaaatcctgaatgtgaaagcctgtctacagccagcagctggtcttatatcgtggaaacccctagcagcgacaatggcacctgttaccctggcgacttcatcgattacgaggagctgagagaacagctgtctagcgtgtccagcttcgagagattcgagatcttccctaagacaagcagctggcctaatcacgattctaataagggagtgacagccgcctgtcctcatgccggagccaagtccttttacaagaacctgatctggctggtgaagaagggcaacagctaccctaagctgtctaagagctacatcaacgacaagggcaaagaagtgctggtgctgtggggaatccaccaccctagcacaagcgccgatcagcagagcctgtaccagaatgccgatgcctatgtgtttgtgggcagcagcagatacagcaaaaagttcaagccttccctgctgaccgaggtggagacccccaccaggaacggctgggagtgcaagtgctccgactccggcagaatgaattactactggaccctggtggaacctggcgataagatcacatttgaggccaccggaaatctggtggtgcctagatatgcatttgctatggagagaaatgctggctctggcatcattatctctgatacccctgtgcacgactgtaataccacctgtcagacacctaagggcgccattaataccagcctgcccttccagaatattcaccctatcaccatcggcaagtgtcctaagtatgtgaagagcaccaagctgagactggctaccggtctgagaaatagccctgaaaacctgtattttcaaggcctgtttggagccatcgccggctttattgagggaggatggaccggaatggtggatggctggtacggctatcaccaccagaatgagcagggatccggatatgccgccgatctgaagtctacacagaacgccatcgacgagatcacaaacaaggtgaacagcgtgatcgagaagatgaacacccagtttacagctgtgggcaaggagttcaaccacctggagaagagaatcgagaacctgaacaagaaagtggacgacggcttcctggatatttggacctacaatgccgagctgctcgtgctcctggagaatgagagaaccctggactaccacgacagcaatgtgaagaacctgtacgagaaggtgagaagccagctgaagaacaatgccaaggagatcggcaacggctgctttgagttctaccacaagtgtgacaacacctgtatggagtctgtgaagaacggcacctacgactaccctaagtatagcgaggaggccaagctgaatagagaggagatcgacggcgtgaaactggaaagcacaagaatctatcagggcgctgaaaacctgtattttcagggcggttctggttacatcccggaagctccgcgtgacggtcaggcttacgttcgtaaagacggtgaatgggttctgctgtctaccttcctgggtcaccatcatcaccaccatcaccatcatcactgataaaagctt